European Patent Application EP 4 796 130 A1, published August 26, 2026. Title: Anti-Tissue Factor Antibody-Drug Conjugates Containing Camptothecin Derivatives. Applicant: CELLTRION, INC. The sequence listing filed with the application follows.

SEQUENCE LISTING (12 sequences)

SEQ ID NO: 1 - protein, 8 aa, synthetic construct
GFTFSNYA

SEQ ID NO: 2 - protein, 8 aa, synthetic construct
ISGSGDYT

SEQ ID NO: 3 - protein, 11 aa, synthetic construct
ARSPWGYYLDS

SEQ ID NO: 4 - protein, 6 aa, synthetic construct
QGISSR

SEQ ID NO: 5 - skipped

SEQ ID NO: 6 - protein, 9 aa, synthetic construct
QQYNSYPYT

SEQ ID NO: 7 - protein, 118 aa, synthetic construct
EVQLLESGGGLVQPGGSLRLSCAASGFTFSNYAMSWVRQAPGKGLEWVSSISGSGDYTYYTDSVKGRFTISRDNSKNTLYLQMNSLRAEDTAVYYCARSPWGYYLDSWGQGTLVTVSS

SEQ ID NO: 8 - protein, 107 aa, synthetic construct
DIQMTQSPPSLSASAGDRVTITCRASQGISSRLAWYQQKPEKAPKSLIYAASSLQSGVPSRFSGSGSGTDFTLTISSLQPEDFATYYCQQYNSYPYTFGQGTKLEIK

SEQ ID NO: 9 - protein, 448 aa, synthetic construct
EVQLLESGGGLVQPGGSLRLSCAASGFTFSNYAMSWVRQAPGKGLEWVSSISGSGDYTYYTDSVKGRFTISRDNSKNTLYLQMNSLRAEDTAVYYCARSPWGYYLDSWGQGTLVTVSSASTKGPSVFPLAPSSKSTSGGTAALGCLVKDYFPEPVTVSWNSGALTSGVHTFPAVLQSSGLYSLSSVVTVPSSSLGTQTYICNVNHKPSNTKVDKKVEPKSCDKTHTCPPCPAPELLGGPSVFLFPPKPKDTLMISRTPEVTCVVVDVSHEDPEVKFNWYVDGVEVHNAKTKPREEQYNSTYRVVSVLTVLHQDWLNGKEYKCKVSNKALPAPIEKTISKAKGQPREPQVYTLPPSRDELTKNQVSLTCLVKGFYPSDIAVEWESNGQPENNYKTTPPVLDSDGSFFLYSKLTVDKSRWQQGNVFSCSVMHEALHNHYTQKSLSLSPGK

SEQ ID NO: 10 - protein, 214 aa, synthetic construct
DIQMTQSPPSLSASAGDRVTITCRASQGISSRLAWYQQKPEKAPKSLIYAASSLQSGVPSRFSGSGSGTDFTLTISSLQPEDFATYYCQQYNSYPYTFGQGTKLEIKRTVAAPSVFIFPPSDEQLKSGTASVVCLLNNFYPREAKVQWKVDNALQSGNSQESVTEQDSKDSTYSLSSTLTLSKADYEKHKVYACEVTHQGLSSPVTKSFNRGEC

SEQ ID NO: 11 - protein, 475 aa, synthetic construct
MDWTWSILFLVAAATGAHSQVQLVQSGAEVKKPGASVKVSCKTSGYSFSTYGVSWVRQAPGQGPEWVGWISAYTGITDYAQKFQGRVTLTTDATTATAFLDLRSLRPDDTATYFCARDKVQGRVEVGSGGRHDYWGQGTLVIVSSASTKGPSVFPLAPSSKSTSGGTAALGCLVKDYFPEPVTVSWNSGALTSGVHTFPAVLQSSGLYSLSSVVTVPSSSLGTQTYICNVNHKPSNTKVDKKVEPKSCDKTHTCPPCPAPELLGGPSVFLFPPKPKDTLMISRTPEVTCVVVDVSHEDPEVKFNWYVDGVEVHNAKTKPREEQYNSTYRVVSVLTVLHQDWLNGKEYKCKVSNKALPAPIEKTISKAKGQPREPQVYTLPPSRDELTKNQVSLTCLVKGFYPSDIAVEWESNGQPENNYKTTPPVLDSDGSFFLYSKLTVDKSRWQQGNVFSCSVMHEGLHNHYTQKSLSLSPGK

SEQ ID NO: 12 - protein, 235 aa, synthetic construct
METPAQLLFLLLLWLPDTTGEVVLTQSPGTLALPPGERATLSCRASHRVGSTYIAWYQQKSGQAPRRLIYGASNRATDIPDRFSGSGSGTDFTLTIRRLEPEDSAVYYCQQFSVSPWTFGQGTRVEIKRTVAAPSVFIFPPSDEQLKSGTASVVCLLNNFYPREAKVQWKVDNALQSGNSQESVTEQDSKDSTYSLSSTLTLSKADYEKHKVYACEVTHQGLSSPVTKSFNRGEC